European Patent Specification EP 3 971 212 B1, published December 27, 2023. Title: ONCOSTATIN M RECEPTOR ANTIGEN BINDING PROTEINS. Applicant: KINIKSA PHARMACEUTICALS, LTD. Arnett, et al. The sequence listing filed with the application follows.

SEQUENCE LISTING (54 sequences)

SEQ ID NO: 1 - protein, 979 aa, Homo sapiens
  source: /note="Human OSMR"
MALFAVFQTTFFLTLLSLRTYQSEVLAERLPLTPVSLKVSTNSTRQSLHLQWTVHNLPYHQELKMVFQIQISRIETSNVIWVGNYSTTVKWNQVLHWSWESELPLECATHFVRIKSLVDDAKFPEPNFWSNWSSWEEVSVQDSTGQDILFVFPKDKLVEEGTNVTICYVSRNIQNNVSCYLEGKQIHGEQLDPHVTAFNLNSVPFIRNKGTNIYCEASQGNVSEGMKGIVLFVSKVLEEPKDFSCETEDFKTLHCTWDPGTDTALGWSKQPSQSYTLFESFSGEKKLCTHKNWCNWQITQDSQETYNFTLIAENYLRKRSVNILFNLTHRVYLMNPFSVNFENVNATNAIMTWKVHSIRNNFTYLCQIELHGEGKMMQYNVSIKVNGEYFLSELEPATEYMARVRCADASHFWKWSEWSGQNFTTLEAAPSEAPDVWRIVSLEPGNHTVTLFWKPLSKLHANGKILFYNVVVENLDKPSSSELHSIPAPANSTKLILDRCSYQICVIANNSVGASPASVIVISADPENKEVEEERIAGTEGGFSLSWKPQPGDVIGYVVDWCDHTQDVLGDFQWKNVGPNTTSTVISTDAFRPGVRYDFRIYGLSTKRIACLLEKKTGYSQELAPSDNPHVLVDTLTSHSFTLSWKDYSTESQPGFIQGYHVYLKSKARQCHPRFEKAVLSDGSECCKYKIDNPEEKALIVDNLKPESFYEFFITPFTSAGEGPSATFTKVTTPDEHSSMLIHILLPMVFCVLLIMVMCYLKSQWIKETCYPDIPDPYKSSILSLIKFKENPHLIIMNVSDCIPDAIEVVSKPEGTKIQFLGTRKSLTETELTKPNYLYLLPTEKNHSGPGPCICFENLTYNQAASDSGSCGHVPVSPKAPSMLGLMTSPENVLKALEKNYMNSLGEIPAGETSLNYVSQLASPMFGDKDSLPTNPVEAPHCSEYKMQMAVSLRLALPPPTENSSLSSITLLDPGEHYC

SEQ ID NO: 2 - protein, 977 aa, Macaca fascicularis
  source: /note="Cynomolgus monkey OSMR"
MALFVVFQTTFFLILLSLRTYQSEVLAERLPLTPVSLKVSTNSIHQSLHLQWTVHNLPYHQELKMVFQIQISRIETSNVVWVGNYSTPVKWNQVLHWSWESELPLECATHFVRIKSVIDDASFPEPNFWSNWSSWEEVSVQDYLGRGTLFVFPKDKLVEEGSNVTICYVSRNIQNNVSCYLEGKQIHGEQLDPHVTAFNLNSVPFIRNRGTNIYCEASQGNVSKGIEGIVLFVSKVLEEPKDFSCESQDFKTLHCTWDPGTDTALGWSKQPSQSYTLFESFSGEKKLCTHKNWCNWQITQDSQEMYNFTLIAENYLRKRSVNILFNLTHRVYLMNPFSVNFENVNATNAIMTWKVHSMRNNFTYLCQIELHGEGKMMQYDVSINVNGEYFLSELEPATEYMARVRCADASHFWKWTEWSGQNFTTLEAAPSEAPDVWRSVNSEPGNHTVTLFWKPLSKLHANGKILFYNVVVENLDKPSRSELRSIPAPANSTKLILDRCSYQICVTANNSVGASPASIIVISADPENKEVEEERIAGTEGGFSLSWKPQPGDVIGYVVDWCDHPQDVLQWKNVGPNTTSTVISTDAFRPGVRYDFRIYGLSTKRIACLLEKKTGYSQELAPSDNPHVLVDMLTSHSFTLSWKDYSTESQPGFIQGYHVYLKSKARQCHPRFQKAVLSDGSECCRYKIDNPEEKALIVDNLKPESFYEFFVTPFTSAGEGPNATFTKVTTPDEHSSMLIRILLPMVFCVLLIMIVCYLKSQWIKETCYPDIPDPYKSSILSLIKFKENPHLTIMNVSDCIPDAIEVVSKPEGTKIQLLGTRKSLTETELTKPNYLYLLPTEKNHSGPGPCICFENFTYNQAASDAGSCGHVPVPPKAPPSMLGLMTSPENVLKALEKNYMNSLGEVPAGETSLNYVSQLASPMSGDKDSLPTNPVEPPHCSEYKMQMAVPLRLALPPPTENSSLSSITLLDPGEHYR

SEQ ID NO: 3 - DNA, 1356 bp, Homo sapiens
  source: /note="Ab1 Heavy chain"
caggtgcagctggtgcagtctggggctgaggtgaagaagcctggggcctcagtgaaggtctcctgcaaggcttctggatacaccttcaccagttatgatatcaactgggtgcgacaggccactggacaggggcttgagtggatgggatggatgaaccctaatagtggtaacacagactatgcacagaagttccagggcagagtcaccatgaccaggaacatttccataagcacggcctacattgagctgagcagcctgagatctgaggacacggccgtttattactgtgcgagagatatggtggctgcgaatacggattactacttctactacggtatggacgtctggggccaagggaccacggtcaccgtctcctcagctagcaccaagggcccatcggtcttccccctggcgccctgctccaggagcacctccgagagcacagcggccctgggctgcctggtcaaggactacttccccgaaccggtgacggtgtcgtggaactcaggcgctctgaccagcggcgtgcacaccttcccagctgtcctacagtcctcaggactctactccctcagcagcgtggtgaccgtgccctccagcaacttcggcacccagacctacacctgcaacgtagatcacaagcccagcaacaccaaggtggacaagacagttgagcgcaaatgttgtgtcgagtgcccaccgtgcccagcaccacctgtggcaggaccgtcagtcttcctcttccccccaaaacccaaggacaccctcatgatctcccggacccctgaggtcacgtgcgtggtggtggacgtgagccacgaagaccccgaggtccagttcaactggtacgtggacggcgtggaggtgcataatgccaagacaaagccacgggaggagcagttcaacagcacgttccgtgtggtcagcgtcctcaccgttgtgcaccaggactggctgaacggcaaggagtacaagtgcaaggtctccaacaaaggcctcccagcccccatcgagaaaaccatctccaaaaccaaagggcagccccgagaaccacaggtgtacaccctgcccccatcccgggaggagatgaccaagaaccaggtcagcctgacctgcctggtcaaaggcttctaccccagcgacatcgccgtggagtgggagagcaatgggcagccggagaacaactacaagaccacacctcccatgctggactccgacggctccttcttcctctacagcaagctcaccgtggacaagagcaggtggcagcaggggaacgtcttctcatgctccgtgatgcatgaggctctgcacaaccactacacgcagaagagcctctccctgtctccgggtaaa

SEQ ID NO: 4 - DNA, 1356 bp, Homo sapiens
  source: /note="Ab2 Heavy chain"
caggtgcagctggtgcagtctggggctgaggtgaagaagcctggggcctcagtgaaggtctcctgcaaggcttctggatacaccttcaccagttatgaaatcaactgggtgcgacaggccactggacaagggcttgagtggatgggatggatgaaccctaacagtggttacacaggctatgcacagaagttccagggcagagtcaccatgaccaggaacacctccataagcacagcctacatggaaatgagcagcctgagatctgaggacacggccgtgtattactgtgcgagagatatagtggctgcgaatacggattactacttctattatggtatggacgtctggggccaagggaccacggtcaccgtctcctcagctagcaccaagggcccatcggtcttccccctggcgccctgctccaggagcacctccgagagcacagcggccctgggctgcctggtcaaggactacttccccgaaccggtgacggtgtcgtggaactcaggcgctctgaccagcggcgtgcacaccttcccagctgtcctacagtcctcaggactctactccctcagcagcgtggtgaccgtgccctccagcaacttcggcacccagacctacacctgcaacgtagatcacaagcccagcaacaccaaggtggacaagacagttgagcgcaaatgttgtgtcgagtgcccaccgtgcccagcaccacctgtggcaggaccgtcagtcttcctcttccccccaaaacccaaggacaccctcatgatctcccggacccctgaggtcacgtgcgtggtggtggacgtgagccacgaagaccccgaggtccagttcaactggtacgtggacggcgtggaggtgcataatgccaagacaaagccacgggaggagcagttcaacagcacgttccgtgtggtcagcgtcctcaccgttgtgcaccaggactggctgaacggcaaggagtacaagtgcaaggtctccaacaaaggcctcccagcccccatcgagaaaaccatctccaaaaccaaagggcagccccgagaaccacaggtgtacaccctgcccccatcccgggaggagatgaccaagaaccaggtcagcctgacctgcctggtcaaaggcttctaccccagcgacatcgccgtggagtgggagagcaatgggcagccggagaacaactacaagaccacacctcccatgctggactccgacggctccttcttcctctacagcaagctcaccgtggacaagagcaggtggcagcaggggaacgtcttctcatgctccgtgatgcatgaggctctgcacaaccactacacgcagaagagcctctccctgtctccgggtaaa

SEQ ID NO: 5 - DNA, 1335 bp, Homo sapiens
  source: /note="Ab3 Heavy chain"
caggttcatctggtgcagtctggagctgaggtgaagaagcctggggcctcagtgaaggtctcctgcaaggcttctggttacacctttaccagctatggtatcagctgggtgcgacaggcccctggacaagggcttgagtggatgggatggctcagcacttacagtggtaacacaaactatgcacagaagctccagggcagagtcaccatgaccacagacacatccacgagcacagcctacatggagctgaggagcctgagatctgacgacacggccgtgtattactgtgcgagagggaacttctactactacggtatggacgtctggggccaggggaccacggtcaccgtctcctcagctagcaccaagggcccatcggtcttccccctggcgccctgctccaggagcacctccgagagcacagcggccctgggctgcctggtcaaggactacttccccgaaccggtgacggtgtcgtggaactcaggcgctctgaccagcggcgtgcacaccttcccagctgtcctacagtcctcaggactctactccctcagcagcgtggtgaccgtgccctccagcaacttcggcacccagacctacacctgcaacgtagatcacaagcccagcaacaccaaggtggacaagacagttgagcgcaaatgttgtgtcgagtgcccaccgtgcccagcaccacctgtggcaggaccgtcagtcttcctcttccccccaaaacccaaggacaccctcatgatctcccggacccctgaggtcacgtgcgtggtggtggacgtgagccacgaagaccccgaggtccagttcaactggtacgtggacggcgtggaggtgcataatgccaagacaaagccacgggaggagcagttcaacagcacgttccgtgtggtcagcgtcctcaccgttgtgcaccaggactggctgaacggcaaggagtacaagtgcaaggtctccaacaaaggcctcccagcccccatcgagaaaaccatctccaaaaccaaagggcagccccgagaaccacaggtgtacaccctgcccccatcccgggaggagatgaccaagaaccaggtcagcctgacctgcctggtcaaaggcttctaccccagcgacatcgccgtggagtgggagagcaatgggcagccggagaacaactacaagaccacacctcccatgctggactccgacggctccttcttcctctacagcaagctcaccgtggacaagagcaggtggcagcaggggaacgtcttctcatgctccgtgatgcatgaggctctgcacaaccactacacgcagaagagcctctccctgtctccgggtaaa

SEQ ID NO: 6 - protein, 452 aa, Homo sapiens
  source: /note="Ab1 Heavy chain"
QVQLVQSGAEVKKPGASVKVSCKASGYTFTSYDINWVRQATGQGLEWMGWMNPNSGNTDYAQKFQGRVTMTRNISISTAYIELSSLRSEDTAVYYCARDMVAANTDYYFYYGMDVWGQGTTVTVSSASTKGPSVFPLAPCSRSTSESTAALGCLVKDYFPEPVTVSWNSGALTSGVHTFPAVLQSSGLYSLSSVVTVPSSNFGTQTYTCNVDHKPSNTKVDKTVERKCCVECPPCPAPPVAGPSVFLFPPKPKDTLMISRTPEVTCVVVDVSHEDPEVQFNWYVDGVEVHNAKTKPREEQFNSTFRVVSVLTVVHQDWLNGKEYKCKVSNKGLPAPIEKTISKTKGQPREPQVYTLPPSREEMTKNQVSLTCLVKGFYPSDIAVEWESNGQPENNYKTTPPMLDSDGSFFLYSKLTVDKSRWQQGNVFSCSVMHEALHNHYTQKSLSLSPGK

SEQ ID NO: 7 - protein, 452 aa, Homo sapiens
  source: /note="Ab2 Heavy chain"
QVQLVQSGAEVKKPGASVKVSCKASGYTFTSYEINWVRQATGQGLEWMGWMNPNSGYTGYAQKFQGRVTMTRNTSISTAYMEMSSLRSEDTAVYYCARDIVAANTDYYFYYGMDVWGQGTTVTVSSASTKGPSVFPLAPCSRSTSESTAALGCLVKDYFPEPVTVSWNSGALTSGVHTFPAVLQSSGLYSLSSVVTVPSSNFGTQTYTCNVDHKPSNTKVDKTVERKCCVECPPCPAPPVAGPSVFLFPPKPKDTLMISRTPEVTCVVVDVSHEDPEVQFNWYVDGVEVHNAKTKPREEQFNSTFRVVSVLTVVHQDWLNGKEYKCKVSNKGLPAPIEKTISKTKGQPREPQVYTLPPSREEMTKNQVSLTCLVKGFYPSDIAVEWESNGQPENNYKTTPPMLDSDGSFFLYSKLTVDKSRWQQGNVFSCSVMHEALHNHYTQKSLSLSPGK

SEQ ID NO: 8 - protein, 445 aa, Homo sapiens
  source: /note="Ab3 Heavy chain"
QVHLVQSGAEVKKPGASVKVSCKASGYTFTSYGISWVRQAPGQGLEWMGWLSTYSGNTNYAQKLQGRVTMTTDTSTSTAYMELRSLRSDDTAVYYCARGNFYYYGMDVWGQGTTVTVSSASTKGPSVFPLAPCSRSTSESTAALGCLVKDYFPEPVTVSWNSGALTSGVHTFPAVLQSSGLYSLSSVVTVPSSNFGTQTYTCNVDHKPSNTKVDKTVERKCCVECPPCPAPPVAGPSVFLFPPKPKDTLMISRTPEVTCVVVDVSHEDPEVQFNWYVDGVEVHNAKTKPREEQFNSTFRVVSVLTVVHQDWLNGKEYKCKVSNKGLPAPIEKTISKTKGQPREPQVYTLPPSREEMTKNQVSLTCLVKGFYPSDIAVEWESNGQPENNYKTTPPMLDSDGSFFLYSKLTVDKSRWQQGNVFSCSVMHEALHNHYTQKSLSLSPGK

SEQ ID NO: 9 - protein, 126 aa, Homo sapiens
  source: /note="Ab1 Heavy chain variable region"
QVQLVQSGAEVKKPGASVKVSCKASGYTFTSYDINWVRQATGQGLEWMGWMNPNSGNTDYAQKFQGRVTMTRNISISTAYIELSSLRSEDTAVYYCARDMVAANTDYYFYYGMDVWGQGTTVTVSS

SEQ ID NO: 10 - protein, 126 aa, Homo sapiens
  source: /note="Ab2 Heavy chain variable region"
QVQLVQSGAEVKKPGASVKVSCKASGYTFTSYEINWVRQATGQGLEWMGWMNPNSGYTGYAQKFQGRVTMTRNTSISTAYMEMSSLRSEDTAVYYCARDIVAANTDYYFYYGMDVWGQGTTVTVSS

SEQ ID NO: 11 - protein, 119 aa, Homo sapiens
  source: /note="Ab3 Heavy chain variable region"
QVHLVQSGAEVKKPGASVKVSCKASGYTFTSYGISWVRQAPGQGLEWMGWLSTYSGNTNYAQKLQGRVTMTTDTSTSTAYMELRSLRSDDTAVYYCARGNFYYYGMDVWGQGTTVTVSS

SEQ ID NO: 12 - protein, 5 aa, Homo sapiens
  source: /note="Ab1 Heavy chain CDR1"
SYDIN

SEQ ID NO: 13 - protein, 5 aa, Homo sapiens
  source: /note="Ab2 Heavy chain CDR1"
SYEIN

SEQ ID NO: 14 - protein, 5 aa, Homo sapiens
  source: /note="Ab3 Heavy chain CDR1"
SYGIS

SEQ ID NO: 15 - protein, 17 aa, Homo sapiens
  source: /note="Ab1 Heavy chain CDR2"
WMNPNSGNTDYAQKFQG

SEQ ID NO: 16 - protein, 20 aa, Homo sapiens
  source: /note="Ab2 Heavy chain CDR2"
WMGWMNPNSGYTGYAQKFQG

SEQ ID NO: 17 - protein, 17 aa, Homo sapiens
  source: /note="Ab3 Heavy chain CDR2"
WLSTYSGNTNYAQKLQG

SEQ ID NO: 18 - protein, 17 aa, Homo sapiens
  source: /note="Ab1 Heavy chain CDR3"
DMVAANTDYYFYYGMDV

SEQ ID NO: 19 - protein, 17 aa, Homo sapiens
  source: /note="Ab2 Heavy chain CDR3"
DIVAANTDYYFYYGMDV

SEQ ID NO: 20 - protein, 10 aa, Homo sapiens
  source: /note="Ab3 Heavy chain CDR3"
GNFYYYGMDV

SEQ ID NO: 21 - DNA, 648 bp, Homo sapiens
  source: /note="Ab1 Light chain"
cagtctgtgctgactcagccaccctcagcatctgggacccccgggcagagggtcaccatctcttgttctggaagcagctccaacgtcggaagtaatactgtaagctggtaccaacagctcccaggaacggcccccaaactcctcatctatactaataatcggcggccctccggggtccctgaccgattctctggctccaagtctggcacctcagcctccctggccatcagtgggctccagtctgaggatgaggctgattatttctgtgcagcgttagatgacagtctgaatggtgtggtattcggcggagggaccaaactgaccgtcctaggccaaccgaaagcggcgccctcggtcactctgttcccgccctcctctgaggagcttcaagccaacaaggccacactggtgtgtctcataagtgacttctacccgggagccgtgacagtggcctggaaggcagatagcagccccgtcaaggcgggagtggagaccaccacaccctccaaacaaagcaacaacaagtacgcggccagcagctatctgagcctgacgcctgagcagtggaagtcccacagaagctacagctgccaggtcacgcatgaagggagcaccgtggagaagacagtggcccctacagaatgttca

SEQ ID NO: 22 - DNA, 648 bp, Homo sapiens
  source: /note="Ab2 Light chain"
cagtctgtgctgactcagccaccctcagcgtctgggacccccgggcagagggtcaccatctcttgttctggaagcaactccaacatcggaagtaatactgtcaactggtaccaccagctcccaggaacggcccccaaactcctcatctataatattaataagcggccctcaggggtccctgaccgattctctggctccaagtctggctcctcagcctccctggccatcagtgggctccagtctgaggatgaggctgattattactgttcaacatgggatgacagcctggatggtgtggtattcggcggagggaccaagctgaccgtcctaggccaaccgaaagcggcgccctcggtcactctgttcccgccctcctctgaggagcttcaagccaacaaggccacactggtgtgtctcataagtgacttctacccgggagccgtgacagtggcctggaaggcagatagcagccccgtcaaggcgggagtggagaccaccacaccctccaaacaaagcaacaacaagtacgcggccagcagctatctgagcctgacgcctgagcagtggaagtcccacagaagctacagctgccaggtcacgcatgaagggagcaccgtggagaagacagtggcccctacagaatgttca

SEQ ID NO: 23 - DNA, 648 bp, Homo sapiens
  source: /note="Ab3 Light chain"
gaaattgtgttgacgcagtctccaggcaccctgtctttgtctccaggggaaagagccaccctctcctgcagggccagtcagagtgttagcagcagctacttagcctggtaccagcagaaacctggccaggctcccaggctcctcatctttggtgcttccagcagggccactggcatcccagacaggttcagtggcagtgggtctgggacagacttcactctcaccatcagcagactggagcctgaagattttgcagtgtattactgtcagcagtatggtagctcgcctccgatcaccttcggccaagggacacgactggagattaaacgtacggtggctgcaccatctgtcttcatcttcccgccatctgatgagcagttgaaatctggaactgcctctgttgtgtgcctgctgaataacttctatcccagagaggccaaagtacagtggaaggtggataacgccctccaatcgggtaactcccaggagagtgtcacagagcaggacagcaaggacagcacctacagcctcagcagcaccctgacgctgagcaaagcagactacgagaaacacaaagtctacgcctgcgaagtcacccatcagggcctgagctcgcccgtcacaaagagcttcaacaggggagagtgt

SEQ ID NO: 24 - protein, 216 aa, Homo sapiens
  source: /note="Ab1 Light chain"
QSVLTQPPSASGTPGQRVTISCSGSSSNVGSNTVSWYQQLPGTAPKLLIYTNNRRPSGVPDRFSGSKSGTSASLAISGLQSEDEADYFCAALDDSLNGVVFGGGTKLTVLGQPKAAPSVTLFPPSSEELQANKATLVCLISDFYPGAVTVAWKADSSPVKAGVETTTPSKQSNNKYAASSYLSLTPEQWKSHRSYSCQVTHEGSTVEKTVAPTECS

SEQ ID NO: 25 - protein, 216 aa, Homo sapiens
  source: /note="Ab2 Light chain"
QSVLTQPPSASGTPGQRVTISCSGSNSNIGSNTVNWYHQLPGTAPKLLIYNINKRPSGVPDRFSGSKSGSSASLAISGLQSEDEADYYCSTWDDSLDGVVFGGGTKLTVLGQPKAAPSVTLFPPSSEELQANKATLVCLISDFYPGAVTVAWKADSSPVKAGVETTTPSKQSNNKYAASSYLSLTPEQWKSHRSYSCQVTHEGSTVEKTVAPTECS

SEQ ID NO: 26 - protein, 216 aa, Homo sapiens
  source: /note="Ab3 light chain"
EIVLTQSPGTLSLSPGERATLSCRASQSVSSSYLAWYQQKPGQAPRLLIFGASSRATGIPDRFSGSGSGTDFTLTISRLEPEDFAVYYCQQYGSSPPITFGQGTRLEIKRTVAAPSVFIFPPSDEQLKSGTASVVCLLNNFYPREAKVQWKVDNALQSGNSQESVTEQDSKDSTYSLSSTLTLSKADYEKHKVYACEVTHQGLSSPVTKSFNRGEC

SEQ ID NO: 27 - protein, 111 aa, Homo sapiens
  source: /note="Ab1 Light chain variable"
QSVLTQPPSASGTPGQRVTISCSGSSSNVGSNTVSWYQQLPGTAPKLLIYTNNRRPSGVPDRFSGSKSGTSASLAISGLQSEDEADYFCAALDDSLNGVVFGGGTKLTVLG

SEQ ID NO: 28 - protein, 111 aa, Homo sapiens
  source: /note="Ab2 Light chain variable"
QSVLTQPPSASGTPGQRVTISCSGSNSNIGSNTVNWYHQLPGTAPKLLIYNINKRPSGVPDRFSGSKSGSSASLAISGLQSEDEADYYCSTWDDSLDGVVFGGGTKLTVLG

SEQ ID NO: 29 - protein, 110 aa, Homo sapiens
  source: /note="Ab3 Light chain variable"
EIVLTQSPGTLSLSPGERATLSCRASQSVSSSYLAWYQQKPGQAPRLLIFGASSRATGIPDRFSGSGSGTDFTLTISRLEPEDFAVYYCQQYGSSPPITFGQGTRLEIKR

SEQ ID NO: 30 - protein, 13 aa, Homo sapiens
  source: /note="Ab1 Light chain CDR1"
SGSSSNVGSNTVS

SEQ ID NO: 31 - protein, 13 aa, Homo sapiens
  source: /note="Ab2 Light chain CDR1"
SGSNSNIGSNTVN

SEQ ID NO: 32 - protein, 12 aa, Homo sapiens
  source: /note="Ab3 Light chain CDR1"
RASQSVSSSYLA

SEQ ID NO: 33 - protein, 7 aa, Homo sapiens
  source: /note="Ab1 Light chain CDR2"
TNNRRPS

SEQ ID NO: 34 - protein, 7 aa, Homo sapiens
  source: /note="Ab2 Light chain CDR2"
NINKRPS

SEQ ID NO: 35 - protein, 7 aa, Homo sapiens
  source: /note="Ab3 Light chain CDR2"
GASSRAT

SEQ ID NO: 36 - protein, 11 aa, Homo sapiens
  source: /note="Ab1 Light chain CDR3"
AALDDSLNGVV

SEQ ID NO: 37 - protein, 11 aa, Homo sapiens
  source: /note="Ab2 Light chain CDR3"
STWDDSLDGVV

SEQ ID NO: 38 - protein, 10 aa, Homo sapiens
  source: /note="Ab3 Light chain CDR3"
QQYGSSPPIT

SEQ ID NO: 39 - protein, 252 aa, Homo sapiens
  source: /note="Human OSM"
MGVLLTQRTLLSLVLALLFPSMASMAAIGSCSKEYRVLLGQLQKQTDLMQDTSRLLDPYIRIQGLDVPKLREHCRERPGAFPSEETLRGLGRRGFLQTLNATLGCVLHRLADLEQRLPKAQDLERSGLNIEDLEKLQMARPNILGLRNNIYCMAQLLDNSDTAEPTKAGRGASQPPTPTPASDAFQRKLEGCRFLHGYHRFMHSVGRVFSKWGESPNRSRRHSPHQALRKGVRRTRPSRKGKRLMTRGQLPR

SEQ ID NO: 40 - protein, 196 aa, Macaca fascicularis
  source: /note="Cynomolgus monkey OSM protein"
AAMGSCSKEYRMLLGQLQKQTDLMQDTSRLLDPYIRIQGLDIPKLREHCRESPGAFPSEETLRGLGRRGFLQTLNATLGRILHRLADLEQHLPKAQDLERSGLNIEDLEKLQMARPNVLGLRNNVYCMAQLLDNSDMTEPTKAGRGTPQPPTPTPTSDVFQRKLEGCSFLRGYHRFMHSVGRVFSKWGESPNRSRR

SEQ ID NO: 41 - protein, 164 aa, Homo sapiens
  source: /note="Human IL-31"
MASHSGPSTSVLFLFCCLGGWLASHTLPVRLLRPSDDVQKIVEELQSLSKMLLKDVEEEKGVLVSQNYTLPCLSPDAQPPNNIHSPAIRAYLKTIRQLDNKSVIDEIIEHLDKLIFQDAPETNISVPTDTHECKRFILTISQQFSECMDLALKSLTSGAQQATT

SEQ ID NO: 42 - protein, 138 aa, Macaca fascicularis
  source: /note="Cynomolgus monkey IL-31"
TLPVHFLQPSDIQKIVEELQSLSKMLLKDVKEDKGVLVSQNYTLPCLTPDAQPPNIIHSPAIRAYLKTIRQLDNKSVIDEIIEHLDKLIFQDAPETNISVPTDTHECKRFILTISQQFSECMDLALKSLTSGAQQATT

SEQ ID NO: 43 - protein, 662 aa, Homo sapiens
  source: /note="Human IL-31RA"
MKLSPQPSCVNLGMMWTWALWMLPSLCKFSLAALPAKPENISCVYYYRKNLTCTWSPGKETSYTQYTVKRTYAFGEKHDNCTTNSSTSENRASCSFFLPRITIPDNYTIEVEAENGDGVIKSHMTYWRLENIAKTEPPKIFRVKPVLGIKRMIQIEWIKPELAPVSSDLKYTLRFRTVNSTSWMEVNFAKNRKDKNQTYNLTGLQPFTEYVIALRCAVKESKFWSDWSQEKMGMTEEEAPCGLELWRVLKPAEADGRRPVRLLWKKARGAPVLEKTLGYNIWYYPESNTNLTETMNTTNQQLELHLGGESFWVSMISYNSLGKSPVATLRIPAIQEKSFQCIEVMQACVAEDQLVVKWQSSALDVNTWMIEWFPDVDSEPTTLSWESVSQATNWTIQQDKLKPFWCYNISVYPMLHDKVGEPYSIQAYAKEGVPSEGPETKVENIGVKTVTITWKEIPKSERKGIICNYTIFYQAEGGKGFSKTVNSSILQYGLESLKRKTSYIVQVMASTSAGGTNGTSINFKTLSFSVFEIILITSLIGGGLLILIILTVAYGLKKPNKLTHLCWPTVPNPAESSIATWHGDDFKDKLNLKESDDSVNTEDRILKPCSTPSDKLVIDKLVVNFGNVLQEIFTDEARTGQENNLGGEKNGTRILSSCPTSI

SEQ ID NO: 44 - protein, 649 aa, Macaca fascicularis
  source: /note="Cynomolgus monkey IL-21RA"
MMWTWALWMFPLLCKFGLAALPAKPENISCVYYYRKNLTCTWSPGKETSYTQYTAKRTYAFGKKHDNCTTSSSTSENRASCSFFLPRITIPDNYTIEVEAENGDGVIKSDMTCWRLEDIAKTEPPEIFSVKPVLGIKRMIRIEWIKPELAPVSSDLKYALRFRTVNSTSWMEVNFAKNRKDTNQTYNLMGLQAFTEYVVALRCAVKESKFWSDWSQEKMGMTEEEAPCGLELWRVLKPTEVDGRRPVRLLWKKARGAPVLEKTLGYNIWYFPENNTNLTETVNTTNQQLELHLGGESYWVSMISYNSLGKSPVTTLRIPAIQEKSFRCIEVMQACLAEDQLVVKWQSSALDVNTWMIEWFPDMDSEHPTLSWESVSQATNWTIQQDKLKPFWCYNISVYPMLHDKVGEPYSIQAYAKEGIPSKGPETKVENIGVKTVTITWKEIPKSERKGIICNYTIFYQAEGGTGFSKTVNSSILQYGLESLKRKTSYTVRVMASTSAGGINGTSINFKTLSFSVFEIILITSLIGGGLLILIILTVAYGLKKPNKLTHLCWPSVPNPAESSIATWRGDDFKDKLNLKESDDSVNTEDRILKPCSTPSDKLVIDKSVVNFGNVLQEMFTDEARTGQENNLGGEKNENRILSSCPTSI

SEQ ID NO: 45 - protein, 918 aa, Homo sapiens
  source: /note="Human gp130"
MLTLQTWLVQALFIFLTTESTGELLDPCGYISPESPVVQLHSNFTAVCVLKEKCMDYFHVNANYIVWKTNHFTIPKEQYTIINRTASSVTFTDIASLNIQLTCNILTFGQLEQNVYGITIISGLPPEKPKNLSCIVNEGKKMRCEWDGGRETHLETNFTLKSEWATHKFADCKAKRDTPTSCTVDYSTVYFVNIEVWVEAENALGKVTSDHINFDPVYKVKPNPPHNLSVINSEELSSILKLTWTNPSIKSVIILKYNIQYRTKDASTWSQIPPEDTASTRSSFTVQDLKPFTEYVFRIRCMKEDGKGYWSDWSEEASGITYEDRPSKAPSFWYKIDPSHTQGYRTVQLVWKTLPPFEANGKILDYEVTLTRWKSHLQNYTVNATKLTVNLTNDRYLATLTVRNLVGKSDAAVLTIPACDFQATHPVMDLKAFPKDNMLWVEWTTPRESVKKYILEWCVLSDKAPCITDWQQEDGTVHRTYLRGNLAESKCYLITVTPVYADGPGSPESIKAYLKQAPPSKGPTVRTKKVGKNEAVLEWDQLPVDVQNGFIRNYTIFYRTIIGNETAVNVDSSHTEYTLSSLTSDTLYMVRMAAYTDEGGKDGPEFTFTTPKFAQGEIEAIVVPVCLAFLLTTLLGVLFCFNKRDLIKKHIWPNVPDPSKSHIAQWSPHTPPRHNFNSKDQMYSDSNFTDVSVVEIVANDKKPFPEDLKSLDLFKKEKINTEGHSSGIGGSSCMSSSRPSISSSDENESSQNTSSTVQYSTVVHSGYRHQVPSVQVFSRSESTQPLLDSEERPEDLQLVDHVDGGDGILPRQQYFKQNCSQHESSPDISHFERSKQVSSVNEEDFVRLKQQISDHISQSCGSGQMKMFQEVSAADAFGPGTEGQVERFETVGMEAATDEGMPKSYLPQTVRQGGYMPQ

SEQ ID NO: 46 - protein, 918 aa, Macaca fascicularis
  source: /note="Cynomolgus monkey gp130"
MLTLQTWVVQALFIFLTTESIGELLDPCGYISPESPVVQLHSNFTAVCVLKEKCMDYFHVNANYIVWKTNHFTIPKEQYTIINRTASSVTFTDISSLNIQLTCNILTFGQLEQNVYGITIISGLPPEKPKNLSCIVNEGKKMRCEWNRGRETHLETNFTLKSEWATHKFADCKAKRDTPTSCTVDYSTVYFVNIEVWVEAENALGKVTSDHINFDPVYKVKPNPPHNLSVINSEELSSILKLTWTNPSIKSVIRLKYNIQYRTKDASTWSQIPPEDTASTRSSFTVQDLKPFTEYVFRICCMKEDGKGYWSDWSEEANGITYEDRPSKAPSFWYKIDPSHAQGYRTVQLMWKTLPPFEANGKILDYEVTLTRWKSHLQNYTVNDTKLTVNLTNDRYVATLTARNLVGKSDAAVLTIPACDFQATHPVMDLKAFPKDNMLWVEWTTPRESVKKYILEWCVLSDKAPCIADWQQEDGTVHRTHLRGNLAESKCYLITVTPVYADGPGSPESIKAYLKQAPPSKGPTVRTKKVGKNEAVLEWDQLPVDVQNGFIRNYTIFYRTIIGNETAVNVDSSHTEYTLSSLTSDTLYMVRMAAYTDEGGKDGPEFTFTTPKFAQGEIEAIVVPVCLAFLLTTLLGVLFCFNKRDLIKKHIWPNVPDPSKSHIAQWSPHTPPRHNFSSKDQMYSDGNFTDVSVVEIEANDKKPFPEDLKSLDLFKKEKINTEGHSSGIGGSSCMSSSRPSISSSDENESSQNTSSTVQYSTVVHSGYRHQVPSVQVFSRSESTQPLLDSEERPEDLQLVDHVDGSDDILPRQQYFKQNCSQHESSPDISHFERSKQVSSVNEEDFVRLKQQISDHISQSCGSGEMKMFQEVSAADPFGPGTEGQVERFETIGMEAAIDEGMPKSYLPQTVRQGGYMPQ

SEQ ID NO: 47 - DNA, 1353 bp, Artificial Sequence
  source: /note="Description of Artificial Sequence: Synthetic polynucleotide"
caggtgcagctggtgcagtctggggctgaggtgaagaagcctggggcctcagtgaaggtctcctgcaaggcttctggatacaccttcaccagttatgatatcaactgggtgcgacaggccactggacaggggcttgagtggatgggatggatgaaccctaatagtggtaacacagactatgcacagaagttccagggcagagtcaccatgaccagggacatttccataagcacggcctacattgagctgagcagcctgagatctgaggacacggccgtttattactgtgcgagagatatggtggctgcgaatacggattactacttctactacggtatggacgtctggggccaagggaccacggtcaccgtctcctcagctagcaccaagggcccatcggtcttccccctggcgccctgctccaggagcacctccgagagcacagcggccctgggctgcctggtcaaggactacttccccgaaccggtgacggtgtcgtggaactcaggcgctctgaccagcggcgtgcacaccttcccagctgtcctacagtcctcaggactctactccctcagcagcgtggtgaccgtgccctccagcaacttcggcacccagacctacacctgcaacgtagatcacaagcccagcaacaccaaggtggacaagacagttgagcgcaaatgttgtgtcgagtgcccaccgtgcccagcaccacctgtggcaggaccgtcagtcttcctcttccccccaaaacccaaggacaccctcatgatctcccggacccctgaggtcacgtgcgtggtggtggacgtgagccacgaagaccccgaggtccagttcaactggtacgtggacggcgtggaggtgcataatgccaagacaaagccacgggaggagcagttcaacagcacgttccgtgtggtcagcgtcctcaccgttgtgcaccaggactggctgaacggcaaggagtacaagtgcaaggtctccaacaaaggcctcccagcccccatcgagaaaaccatctccaaaaccaaagggcagccccgagaaccacaggtgtacaccctgcccccatcccgggaggagatgaccaagaaccaggtcagcctgacctgcctggtcaaaggcttctaccccagcgacatcgccgtggagtgggagagcaatgggcagccggagaacaactacaagaccacacctcccatgctggactccgacggctccttcttcctctacagcaagctcaccgtggacaagagcaggtggcagcaggggaacgtcttctcatgctccgtgatgcatgaggctctgcacaaccactacacgcagaagagcctctccctgtctccgggt

SEQ ID NO: 48 - DNA, 1353 bp, Artificial Sequence
  source: /note="Description of Artificial Sequence: Synthetic polynucleotide"
caggtgcagctggtgcagtctggggctgaggtgaagaagcctggggcctcagtgaaggtctcctgcaaggcttctggatacaccttcaccagttatgaaatcaactgggtgcgacaggccactggacaagggcttgagtggatgggatggatgaaccctaacagtggttacacaggctatgcacagaagttccagggcagagtcaccatgaccagggacacctccataagcacagcctacatggaaatgagcagcctgagatctgaggacacggccgtgtattactgtgcgagagatatagtggctgcgaatacggattactacttctattatggtatggacgtctggggccaagggaccacggtcaccgtctcctcagctagcaccaagggcccatcggtcttccccctggcgccctgctccaggagcacctccgagagcacagcggccctgggctgcctggtcaaggactacttccccgaaccggtgacggtgtcgtggaactcaggcgctctgaccagcggcgtgcacaccttcccagctgtcctacagtcctcaggactctactccctcagcagcgtggtgaccgtgccctccagcaacttcggcacccagacctacacctgcaacgtagatcacaagcccagcaacaccaaggtggacaagacagttgagcgcaaatgttgtgtcgagtgcccaccgtgcccagcaccacctgtggcaggaccgtcagtcttcctcttccccccaaaacccaaggacaccctcatgatctcccggacccctgaggtcacgtgcgtggtggtggacgtgagccacgaagaccccgaggtccagttcaactggtacgtggacggcgtggaggtgcataatgccaagacaaagccacgggaggagcagttcaacagcacgttccgtgtggtcagcgtcctcaccgttgtgcaccaggactggctgaacggcaaggagtacaagtgcaaggtctccaacaaaggcctcccagcccccatcgagaaaaccatctccaaaaccaaagggcagccccgagaaccacaggtgtacaccctgcccccatcccgggaggagatgaccaagaaccaggtcagcctgacctgcctggtcaaaggcttctaccccagcgacatcgccgtggagtgggagagcaatgggcagccggagaacaactacaagaccacacctcccatgctggactccgacggctccttcttcctctacagcaagctcaccgtggacaagagcaggtggcagcaggggaacgtcttctcatgctccgtgatgcatgaggctctgcacaaccactacacgcagaagagcctctccctgtctccgggt

SEQ ID NO: 49 - DNA, 1332 bp, Artificial Sequence
  source: /note="Description of Artificial Sequence: Synthetic polynucleotide"
caggttcatctggtgcagtctggagctgaggtgaagaagcctggggcctcagtgaaggtctcctgcaaggcttctggttacacctttaccagctatggtatcagctgggtgcgacaggcccctggacaagggcttgagtggatgggatggctcagcacttacagtggtaacacaaactatgcacagaagctccagggcagagtcaccatgaccacagacacatccacgagcacagcctacatggagctgaggagcctgagatctgacgacacggccgtgtattactgtgcgagagggaacttctactactacggtatggacgtctggggccaggggaccacggtcaccgtctcctcagctagcaccaagggcccatcggtcttccccctggcgccctgctccaggagcacctccgagagcacagcggccctgggctgcctggtcaaggactacttccccgaaccggtgacggtgtcgtggaactcaggcgctctgaccagcggcgtgcacaccttcccagctgtcctacagtcctcaggactctactccctcagcagcgtggtgaccgtgccctccagcaacttcggcacccagacctacacctgcaacgtagatcacaagcccagcaacaccaaggtggacaagacagttgagcgcaaatgttgtgtcgagtgcccaccgtgcccagcaccacctgtggcaggaccgtcagtcttcctcttccccccaaaacccaaggacaccctcatgatctcccggacccctgaggtcacgtgcgtggtggtggacgtgagccacgaagaccccgaggtccagttcaactggtacgtggacggcgtggaggtgcataatgccaagacaaagccacgggaggagcagttcaacagcacgttccgtgtggtcagcgtcctcaccgttgtgcaccaggactggctgaacggcaaggagtacaagtgcaaggtctccaacaaaggcctcccagcccccatcgagaaaaccatctccaaaaccaaagggcagccccgagaaccacaggtgtacaccctgcccccatcccgggaggagatgaccaagaaccaggtcagcctgacctgcctggtcaaaggcttctaccccagcgacatcgccgtggagtgggagagcaatgggcagccggagaacaactacaagaccacacctcccatgctggactccgacggctccttcttcctctacagcaagctcaccgtggacaagagcaggtggcagcaggggaacgtcttctcatgctccgtgatgcatgaggctctgcacaaccactacacgcagaagagcctctccctgtctccgggt

SEQ ID NO: 50 - protein, 451 aa, Artificial Sequence
  source: /note="Description of Artificial Sequence: Synthetic polypeptide"
QVQLVQSGAEVKKPGASVKVSCKASGYTFTSYDINWVRQATGQGLEWMGWMNPNSGNTDYAQKFQGRVTMTRDISISTAYIELSSLRSEDTAVYYCARDMVAANTDYYFYYGMDVWGQGTTVTVSSASTKGPSVFPLAPCSRSTSESTAALGCLVKDYFPEPVTVSWNSGALTSGVHTFPAVLQSSGLYSLSSVVTVPSSNFGTQTYTCNVDHKPSNTKVDKTVERKCCVECPPCPAPPVAGPSVFLFPPKPKDTLMISRTPEVTCVVVDVSHEDPEVQFNWYVDGVEVHNAKTKPREEQFNSTFRVVSVLTVVHQDWLNGKEYKCKVSNKGLPAPIEKTISKTKGQPREPQVYTLPPSREEMTKNQVSLTCLVKGFYPSDIAVEWESNGQPENNYKTTPPMLDSDGSFFLYSKLTVDKSRWQQGNVFSCSVMHEALHNHYTQKSLSLSPG

SEQ ID NO: 51 - protein, 451 aa, Artificial Sequence
  source: /note="Description of Artificial Sequence: Synthetic polypeptide"
QVQLVQSGAEVKKPGASVKVSCKASGYTFTSYEINWVRQATGQGLEWMGWMNPNSGYTGYAQKFQGRVTMTRDTSISTAYMEMSSLRSEDTAVYYCARDIVAANTDYYFYYGMDVWGQGTTVTVSSASTKGPSVFPLAPCSRSTSESTAALGCLVKDYFPEPVTVSWNSGALTSGVHTFPAVLQSSGLYSLSSVVTVPSSNFGTQTYTCNVDHKPSNTKVDKTVERKCCVECPPCPAPPVAGPSVFLFPPKPKDTLMISRTPEVTCVVVDVSHEDPEVQFNWYVDGVEVHNAKTKPREEQFNSTFRVVSVLTVVHQDWLNGKEYKCKVSNKGLPAPIEKTISKTKGQPREPQVYTLPPSREEMTKNQVSLTCLVKGFYPSDIAVEWESNGQPENNYKTTPPMLDSDGSFFLYSKLTVDKSRWQQGNVFSCSVMHEALHNHYTQKSLSLSPG

SEQ ID NO: 52 - protein, 444 aa, Artificial Sequence
  source: /note="Description of Artificial Sequence: Synthetic polypeptide"
QVHLVQSGAEVKKPGASVKVSCKASGYTFTSYGISWVRQAPGQGLEWMGWLSTYSGNTNYAQKLQGRVTMTTDTSTSTAYMELRSLRSDDTAVYYCARGNFYYYGMDVWGQGTTVTVSSASTKGPSVFPLAPCSRSTSESTAALGCLVKDYFPEPVTVSWNSGALTSGVHTFPAVLQSSGLYSLSSVVTVPSSNFGTQTYTCNVDHKPSNTKVDKTVERKCCVECPPCPAPPVAGPSVFLFPPKPKDTLMISRTPEVTCVVVDVSHEDPEVQFNWYVDGVEVHNAKTKPREEQFNSTFRVVSVLTVVHQDWLNGKEYKCKVSNKGLPAPIEKTISKTKGQPREPQVYTLPPSREEMTKNQVSLTCLVKGFYPSDIAVEWESNGQPENNYKTTPPMLDSDGSFFLYSKLTVDKSRWQQGNVFSCSVMHEALHNHYTQKSLSLSPG

SEQ ID NO: 53 - protein, 126 aa, Artificial Sequence
  source: /note="Description of Artificial Sequence: Synthetic polypeptide"
QVQLVQSGAEVKKPGASVKVSCKASGYTFTSYDINWVRQATGQGLEWMGWMNPNSGNTDYAQKFQGRVTMTRDISISTAYIELSSLRSEDTAVYYCARDMVAANTDYYFYYGMDVWGQGTTVTVSS

SEQ ID NO: 54 - protein, 126 aa, Artificial Sequence
  source: /note="Description of Artificial Sequence: Synthetic polypeptide"
QVQLVQSGAEVKKPGASVKVSCKASGYTFTSYEINWVRQATGQGLEWMGWMNPNSGYTGYAQKFQGRVTMTRDTSISTAYMEMSSLRSEDTAVYYCARDIVAANTDYYFYYGMDVWGQGTTVTVSS